European Patent Application EP 4 596 043 A2, published August 6, 2025. Title: A LEPTIN RECEPTOR AGONIST ANTIBODY FOR USE IN INCREASING BONE MASS IN A SUBJECT SUFFERING FROM METABOLIC DYSFUNCTION OR HYPOLEPTINEMIA. Applicant: REGENERON PHARMACEUTICALS, INC. Application EP, filed April 5, 2019. The sequence listing filed with the application follows.

SEQUENCE LISTING (120 sequences)

SEQ ID NO: 1 - DNA, 357 bp, synthetic construct
  misc_feature 1..357: note = synthetic
  source 1..357: mol_type = other DNA
caggtgcagctggtggagtctgggggaggcgtggtccagcctgggaagtccctgagactctcctgtgtagcgtctggattcaccttcagttccgatgccatgtactgggtccgccaggctccaggcaaggggctggaatgggtggcagttatttattatgatggaaattatcaatactatgaagactccgttaagggtcgattcaccatctccagagacaattcccagaacacgctggatctgcaaatgaacagcctgagagtcgacgacacggctgtatatttctgtgcgcgtctcaactgggattactggtatctcgatctctggggccgtggcaccctggtcactgtctcctca

SEQ ID NO: 2 - protein, 119 aa, synthetic construct
  REGION 1..119: note = synthetic
QVQLVESGGGVVQPGKSLRLSCVASGFTFSSDAMYWVRQAPGKGLEWVAVIYYDGNYQYYEDSVKGRFTISRDNSQNTLDLQMNSLRVDDTAVYFCARLNWDYWYLDLWGRGTLVTVSS

SEQ ID NO: 3 - DNA, 24 bp, synthetic construct
  misc_feature 1..24: note = synthetic
  source 1..24: mol_type = other DNA
ggattcaccttcagttccgatgcc

SEQ ID NO: 4 - protein, 8 aa, synthetic construct
  REGION 1..8: note = synthetic
GFTFSSDA

SEQ ID NO: 5 - DNA, 24 bp, synthetic construct
  misc_feature 1..24: note = synthetic
  source 1..24: mol_type = other DNA
atttattatgatggaaattatcaa

SEQ ID NO: 6 - protein, 8 aa, synthetic construct
  REGION 1..8: note = synthetic
IYYDGNYQ

SEQ ID NO: 7 - DNA, 36 bp, synthetic construct
  misc_feature 1..36: note = synthetic
  source 1..36: mol_type = other DNA
gcgcgtctcaactgggattactggtatctcgatctc

SEQ ID NO: 8 - protein, 12 aa, synthetic construct
  REGION 1..12: note = synthetic
ARLNWDYWYLDL

SEQ ID NO: 9 - DNA, 324 bp, synthetic construct
  misc_feature 1..324: note = synthetic
  source 1..324: mol_type = other DNA
gacatccagatgacccagtctccatcctccctgtctgcatctgtaggagacagagtcaccatcacttgccgggcaagtcagagcattagcagctatttaaattggtatcagcagaaaccagggaaagcccctaagctcctgatctatgctgcatccagtttgcaaagtggggtcccgtcaaggttcagtggcagtggatctgggacagatttcactctcaccatcagcagtctgcaacctgaagattttgcaacttactactgtcaacagagttacagtacccctccgatcaccttcggccaagggacacgactggagattaaa

SEQ ID NO: 10 - protein, 108 aa, synthetic construct
  REGION 1..108: note = synthetic
DIQMTQSPSSLSASVGDRVTITCRASQSISSYLNWYQQKPGKAPKLLIYAASSLQSGVPSRFSGSGSGTDFTLTISSLQPEDFATYYCQQSYSTPPITFGQGTRLEIK

SEQ ID NO: 11 - DNA, 18 bp, synthetic construct
  misc_feature 1..18: note = synthetic
  source 1..18: mol_type = other DNA
cagagcattagcagctat

SEQ ID NO: 12 - protein, 6 aa, synthetic construct
  REGION 1..6: note = synthetic
QSISSY

SEQ ID NO: 13-14 - skipped (2 entries)

SEQ ID NO: 15 - DNA, 30 bp, synthetic construct
  misc_feature 1..30: note = synthetic
  source 1..30: mol_type = other DNA
caacagagttacagtacccctccgatcacc

SEQ ID NO: 16 - protein, 10 aa, synthetic construct
  REGION 1..10: note = synthetic
QQSYSTPPIT

SEQ ID NO: 17 - DNA, 357 bp, synthetic construct
  misc_feature 1..357: note = synthetic
  source 1..357: mol_type = other DNA
caggtgcagctggtggagtccgggggaggcgtggtccagcctgggaggtccctgagactctcctgtacagcgtctggattcaccttcagtagttatgccatgtactgggtccgccaggctccaggcaaggggctggagtgggtgtcagttatatactatgatggaagttataaatactatgcagactccgtgaagggccgattcaccatctccagagacaattccaagaacacgctgtatctgcaaatggacagcctgagagccgaggacacggctgtctattactgtgcgagttataactggaactactggtacttcgatttctggggccgtggcaccctggtcactgtctcctca

SEQ ID NO: 18 - protein, 119 aa, synthetic construct
  REGION 1..119: note = synthetic
QVQLVESGGGVVQPGRSLRLSCTASGFTFSSYAMYWVRQAPGKGLEWVSVIYYDGSYKYYADSVKGRFTISRDNSKNTLYLQMDSLRAEDTAVYYCASYNWNYWYFDFWGRGTLVTVSS

SEQ ID NO: 19 - DNA, 24 bp, synthetic construct
  misc_feature 1..24: note = synthetic
  source 1..24: mol_type = other DNA
ggattcaccttcagtagttatgcc

SEQ ID NO: 20 - protein, 8 aa, synthetic construct
  REGION 1..8: note = synthetic
GFTFSSYA

SEQ ID NO: 21 - DNA, 24 bp, synthetic construct
  misc_feature 1..24: note = synthetic
  source 1..24: mol_type = other DNA
atatactatgatggaagttataaa

SEQ ID NO: 22 - protein, 8 aa, synthetic construct
  REGION 1..8: note = synthetic
IYYDGSYK

SEQ ID NO: 23 - DNA, 36 bp, synthetic construct
  misc_feature 1..36: note = synthetic
  source 1..36: mol_type = other DNA
gcgagttataactggaactactggtacttcgatttc

SEQ ID NO: 24 - protein, 12 aa, synthetic construct
  REGION 1..12: note = synthetic
ASYNWNYWYFDF

SEQ ID NO: 25 - DNA, 357 bp, synthetic construct
  misc_feature 1..357: note = synthetic
  source 1..357: mol_type = other DNA
caggtgcagctggtggagtctgggggaagcgtggtccagcctgggaggtccctgagactctcctgtgcagcgtctggattcaccttcagtacatatgccatgtactgggtccgccagactccaggcaaggggctggagtgggtggctgttttatactctgatggaagtaataaatactatatagactccgtgaagggccgattcaccatctccagagacacttccacgaacactctgtatctgcaaatgagcagcctgcgagccgacgactcggctctatattactgtgcgcgtctcaactgggattactggtacttcgatctctggggccgtggcaccctggtcactgtctcctca

SEQ ID NO: 26 - protein, 119 aa, synthetic construct
  REGION 1..119: note = synthetic
QVQLVESGGSVVQPGRSLRLSCAASGFTFSTYAMYWVRQTPGKGLEWVAVLYSDGSNKYYIDSVKGRFTISRDTSTNTLYLQMSSLRADDSALYYCARLNWDYWYFDLWGRGTLVTVSS

SEQ ID NO: 27 - DNA, 24 bp, synthetic construct
  misc_feature 1..24: note = synthetic
  source 1..24: mol_type = other DNA
ggattcaccttcagtacatatgcc

SEQ ID NO: 28 - protein, 8 aa, synthetic construct
  REGION 1..8: note = synthetic
GFTFSTYA

SEQ ID NO: 29 - DNA, 24 bp, synthetic construct
  misc_feature 1..24: note = synthetic
  source 1..24: mol_type = other DNA
ttatactctgatggaagtaataaa

SEQ ID NO: 30 - protein, 8 aa, synthetic construct
  REGION 1..8: note = synthetic
LYSDGSNK

SEQ ID NO: 31 - DNA, 36 bp, synthetic construct
  misc_feature 1..36: note = synthetic
  source 1..36: mol_type = other DNA
gcgcgtctcaactgggattactggtacttcgatctc

SEQ ID NO: 32 - protein, 12 aa, synthetic construct
  REGION 1..12: note = synthetic
ARLNWDYWYFDL

SEQ ID NO: 33 - DNA, 357 bp, synthetic construct
  misc_feature 1..357: note = synthetic
  source 1..357: mol_type = other DNA
caggtgcagctggtggagtctgggggaggcgtggtccagcctgggaggtccctgagactctcctgtgaagcgtctggattcagcagcagtgacaatgccatgtactgggtccgccaggctccaggcaaggggctggagtgggtgtcagttatatatcatgatggaagttataaatactatgaagactccgtgaagggccgattcaccatcgccagagacaattccaagaacacgctttatttgcaaatgaacagcctgagagccgaggacacggctgtatattactgtgcgaggtataactggaaccactggtacttcgatgtctggggccgtggcaccctggtcactgtctcctca

SEQ ID NO: 34 - protein, 119 aa, synthetic construct
  REGION 1..119: note = synthetic
QVQLVESGGGVVQPGRSLRLSCEASGFSSSDNAMYWVRQAPGKGLEWVSVIYHDGSYKYYEDSVKGRFTIARDNSKNTLYLQMNSLRAEDTAVYYCARYNWNHWYFDVWGRGTLVTVSS

SEQ ID NO: 35 - DNA, 24 bp, synthetic construct
  misc_feature 1..24: note = synthetic
  source 1..24: mol_type = other DNA
ggattcagcagcagtgacaatgcc

SEQ ID NO: 36 - protein, 8 aa, synthetic construct
  REGION 1..8: note = synthetic
GFSSSDNA

SEQ ID NO: 37 - DNA, 24 bp, synthetic construct
  misc_feature 1..24: note = synthetic
  source 1..24: mol_type = other DNA
atatatcatgatggaagttataaa

SEQ ID NO: 38 - protein, 8 aa, synthetic construct
  REGION 1..8: note = synthetic
IYHDGSYK

SEQ ID NO: 39 - DNA, 36 bp, synthetic construct
  misc_feature 1..36: note = synthetic
  source 1..36: mol_type = other DNA
gcgaggtataactggaaccactggtacttcgatgtc

SEQ ID NO: 40 - protein, 12 aa, synthetic construct
  REGION 1..12: note = synthetic
ARYNWNHWYFDV

SEQ ID NO: 41 - DNA, 366 bp, synthetic construct
  misc_feature 1..366: note = synthetic
  source 1..366: mol_type = other DNA
caggtgcagctggtggagtctgggggaggcgtggtccagcctgggaggtccctgagactctcctgtgcagcctctggattcaccttcagtacctatggcatgcactgggtccgccaggctccaggcaaggggctggagtgggtgtcagttatatcatatgacgaaagtaataagtactatgcagactccgtgaagggccgattcaccatttctagagacaattccaagaacgcgctgtatttacaaatgaacagcctgagaaatgaggacacggctgtgtattactgtgcgagagatcggccttttggattggttaccggatggttcgacccctggggccagggaaccctggtcaccgtctcctca

SEQ ID NO: 42 - protein, 122 aa, synthetic construct
  REGION 1..122: note = synthetic
QVQLVESGGGVVQPGRSLRLSCAASGFTFSTYGMHWVRQAPGKGLEWVSVISYDESNKYYADSVKGRFTISRDNSKNALYLQMNSLRNEDTAVYYCARDRPFGLVTGWFDPWGQGTLVTVSS

SEQ ID NO: 43 - DNA, 24 bp, synthetic construct
  misc_feature 1..24: note = synthetic
  source 1..24: mol_type = other DNA
ggattcaccttcagtacctatggc

SEQ ID NO: 44 - protein, 8 aa, synthetic construct
  REGION 1..8: note = synthetic
GFTFSTYG

SEQ ID NO: 45 - DNA, 24 bp, synthetic construct
  misc_feature 1..24: note = synthetic
  source 1..24: mol_type = other DNA
atatcatatgacgaaagtaataag

SEQ ID NO: 46 - protein, 8 aa, synthetic construct
  REGION 1..8: note = synthetic
ISYDESNK

SEQ ID NO: 47 - DNA, 45 bp, synthetic construct
  misc_feature 1..45: note = synthetic
  source 1..45: mol_type = other DNA
gcgagagatcggccttttggattggttaccggatggttcgacccc

SEQ ID NO: 48 - protein, 15 aa, synthetic construct
  REGION 1..15: note = synthetic
ARDRPFGLVTGWFDP

SEQ ID NO: 49 - DNA, 360 bp, synthetic construct
  misc_feature 1..360: note = synthetic
  source 1..360: mol_type = other DNA
caggtgcagctggtggagtctgggggaggcgtggtccagcctgggaggtccctgagactctcctgtgcagcgtctggattcagtttcaatacctatggcatgcactgggtccgccaggctccaggcaaggggctggagtgggtgacaattatatggtatgatggaagtattaaatactatgcagactccgtgaagggccgattcaccatctccagagacaattccaagaacacgctgtatctgcaaatgaacagcctgagagccgaggacacggctgtgtattattgtgcgagaggtggatatagtggctacctctactttgactactggggccagggaaccctggtcaccgtctcctca

SEQ ID NO: 50 - protein, 120 aa, synthetic construct
  REGION 1..120: note = synthetic
QVQLVESGGGVVQPGRSLRLSCAASGFSFNTYGMHWVRQAPGKGLEWVTIIWYDGSIKYYADSVKGRFTISRDNSKNTLYLQMNSLRAEDTAVYYCARGGYSGYLYFDYWGQGTLVTVSS

SEQ ID NO: 51 - DNA, 24 bp, synthetic construct
  misc_feature 1..24: note = synthetic
  source 1..24: mol_type = other DNA
ggattcagtttcaatacctatggc

SEQ ID NO: 52 - protein, 8 aa, synthetic construct
  REGION 1..8: note = synthetic
GFSFNTYG

SEQ ID NO: 53 - DNA, 24 bp, synthetic construct
  misc_feature 1..24: note = synthetic
  source 1..24: mol_type = other DNA
atatggtatgatggaagtattaaa

SEQ ID NO: 54 - protein, 8 aa, synthetic construct
  REGION 1..8: note = synthetic
IWYDGSIK

SEQ ID NO: 55 - DNA, 39 bp, synthetic construct
  misc_feature 1..39: note = synthetic
  source 1..39: mol_type = other DNA
gcgagaggtggatatagtggctacctctactttgactac

SEQ ID NO: 56 - protein, 13 aa, synthetic construct
  REGION 1..13: note = synthetic
ARGGYSGYLYFDY

SEQ ID NO: 57 - DNA, 372 bp, synthetic construct
  misc_feature 1..372: note = synthetic
  source 1..372: mol_type = other DNA
caggtgcagctgcaggagtcgggcccaggactggtgaagccttcacagaccctgtccctcacctgcactgtctctggtggctccatcagcagcggtggtgactactggagctggatccgccagctcccagggaagggcctggagtggattgggtacatctattacagtgggagcgcctactataatccgtccctcaagagtcgaggtaccatatcaatagacacgtctaagaaccagttctccctgaagctgacctctgtgactgccgcggacacggccgtatatttctgtgtgaaattacgatttttggagtggttcttggggggctggttcggcccctggggccagggaaccctggtcaccgtctcctca

SEQ ID NO: 58 - protein, 124 aa, synthetic construct
  REGION 1..124: note = synthetic
QVQLQESGPGLVKPSQTLSLTCTVSGGSISSGGDYWSWIRQLPGKGLEWIGYIYYSGSAYYNPSLKSRGTISIDTSKNQFSLKLTSVTAADTAVYFCVKLRFLEWFLGGWFGPWGQGTLVTVSS

SEQ ID NO: 59 - DNA, 30 bp, synthetic construct
  misc_feature 1..30: note = synthetic
  source 1..30: mol_type = other DNA
ggtggctccatcagcagcggtggtgactac

SEQ ID NO: 60 - protein, 10 aa, synthetic construct
  REGION 1..10: note = synthetic
GGSISSGGDY

SEQ ID NO: 61 - DNA, 21 bp, synthetic construct
  misc_feature 1..21: note = synthetic
  source 1..21: mol_type = other DNA
atctattacagtgggagcgcc

SEQ ID NO: 62 - protein, 7 aa, synthetic construct
  REGION 1..7: note = synthetic
IYYSGSA

SEQ ID NO: 63 - DNA, 48 bp, synthetic construct
  misc_feature 1..48: note = synthetic
  source 1..48: mol_type = other DNA
gtgaaattacgatttttggagtggttcttggggggctggttcggcccc

SEQ ID NO: 64 - protein, 16 aa, synthetic construct
  REGION 1..16: note = synthetic
VKLRFLEWFLGGWFGP

SEQ ID NO: 65 - DNA, 351 bp, synthetic construct
  misc_feature 1..351: note = synthetic
  source 1..351: mol_type = other DNA
gaggtgcagctggtggagtctgggggaggcttggtacagccgggggggtccctgagactctcctgtgcagcctctggattcacctttagcaactatggcatgacctgggtccgccaggctccagggaagggcctggaatgggtctcagctattactggtggtggtggtagcacatactactcaaactccgtgaagggccggttcaccatctccagagacaattccaagaacacggtgtatctgcgaatgaacagtgtgagagccgaggacacggccgtatattactgtgcgaaatataagtggaacttcgtggacgactggggccagggaaccacggtcaccgtctcctca

SEQ ID NO: 66 - protein, 117 aa, synthetic construct
  REGION 1..117: note = synthetic
EVQLVESGGGLVQPGGSLRLSCAASGFTFSNYGMTWVRQAPGKGLEWVSAITGGGGSTYYSNSVKGRFTISRDNSKNTVYLRMNSVRAEDTAVYYCAKYKWNFVDDWGQGTTVTVSS

SEQ ID NO: 67 - DNA, 24 bp, synthetic construct
  misc_feature 1..24: note = synthetic
  source 1..24: mol_type = other DNA
ggattcacctttagcaactatggc

SEQ ID NO: 68 - protein, 8 aa, synthetic construct
  REGION 1..8: note = synthetic
GFTFSNYG

SEQ ID NO: 69 - DNA, 24 bp, synthetic construct
  misc_feature 1..24: note = synthetic
  source 1..24: mol_type = other DNA
attactggtggtggtggtagcaca

SEQ ID NO: 70 - protein, 8 aa, synthetic construct
  REGION 1..8: note = synthetic
ITGGGGST

SEQ ID NO: 71 - DNA, 30 bp, synthetic construct
  misc_feature 1..30: note = synthetic
  source 1..30: mol_type = other DNA
gcgaaatataagtggaacttcgtggacgac

SEQ ID NO: 72 - protein, 10 aa, synthetic construct
  REGION 1..10: note = synthetic
AKYKWNFVDD

SEQ ID NO: 73 - DNA, 360 bp, synthetic construct
  misc_feature 1..360: note = synthetic
  source 1..360: mol_type = other DNA
gaggtgcagctggtggagtctgggggaggcttggtacagcctggggggtccctgagactctcctgtgttgcctctggattcaccttcaataaatacgacatgcactgggtccgccaaactactggaaaaggtctagagtgggtctcaggtattgatactgatggtgacacatactatccaggctccgtgaagggccgattcaccatctccagagaaaatgccgagaactccctgtatcttcaaatgaacggcctgagagtcggggacacggctgtgtattactgtgcaagatggccttggagtggtttctatggtgcttttgatatctggggccaagggacaatggtcaccgtctcttca

SEQ ID NO: 74 - protein, 120 aa, synthetic construct
  REGION 1..120: note = synthetic
EVQLVESGGGLVQPGGSLRLSCVASGFTFNKYDMHWVRQTTGKGLEWVSGIDTDGDTYYPGSVKGRFTISRENAENSLYLQMNGLRVGDTAVYYCARWPWSGFYGAFDIWGQGTMVTVSS

SEQ ID NO: 75 - DNA, 24 bp, synthetic construct
  misc_feature 1..24: note = synthetic
  source 1..24: mol_type = other DNA
ggattcaccttcaataaatacgac

SEQ ID NO: 76 - protein, 8 aa, synthetic construct
  REGION 1..8: note = synthetic
GFTFNKYD

SEQ ID NO: 77 - DNA, 21 bp, synthetic construct
  misc_feature 1..21: note = synthetic
  source 1..21: mol_type = other DNA
attgatactgatggtgacaca

SEQ ID NO: 78 - protein, 7 aa, synthetic construct
  REGION 1..7: note = synthetic
IDTDGDT

SEQ ID NO: 79 - DNA, 42 bp, synthetic construct
  misc_feature 1..42: note = synthetic
  source 1..42: mol_type = other DNA
gcaagatggccttggagtggtttctatggtgcttttgatatc

SEQ ID NO: 80 - protein, 14 aa, synthetic construct
  REGION 1..14: note = synthetic
ARWPWSGFYGAFDI

SEQ ID NO: 81 - DNA, 366 bp, synthetic construct
  misc_feature 1..366: note = synthetic
  source 1..366: mol_type = other DNA
caggtgcagctgcaggagtcgggcccaggactggtgaagccttcacagaccctgtccctcacctgcactgtctctggtggctccatcagcagtggtaattactactggaactggatccgccaacagccaggagagggcctggagtggattgcttacatctatcacaatggggtcaccaacttcaatccgtccctcaagagtcgacttactatatcagtagacacgtctaagactcagttctccctgaagttgaggtctgtgactgccgcggacacggccgtttattactgtgcgagatcaggcagctggttcgagaactggtacttcgatctctggggccgtggcaccctggtcactgtctcctca

SEQ ID NO: 82 - protein, 122 aa, synthetic construct
  REGION 1..122: note = synthetic
QVQLQESGPGLVKPSQTLSLTCTVSGGSISSGNYYWNWIRQQPGEGLEWIAYIYHNGVTNFNPSLKSRLTISVDTSKTQFSLKLRSVTAADTAVYYCARSGSWFENWYFDLWGRGTLVTVSS

SEQ ID NO: 83 - DNA, 30 bp, synthetic construct
  misc_feature 1..30: note = synthetic
  source 1..30: mol_type = other DNA
ggtggctccatcagcagtggtaattactac

SEQ ID NO: 84 - protein, 10 aa, synthetic construct
  REGION 1..10: note = synthetic
GGSISSGNYY

SEQ ID NO: 85 - DNA, 21 bp, synthetic construct
  misc_feature 1..21: note = synthetic
  source 1..21: mol_type = other DNA
atctatcacaatggggtcacc

SEQ ID NO: 86 - protein, 7 aa, synthetic construct
  REGION 1..7: note = synthetic
IYHNGVT

SEQ ID NO: 87 - DNA, 42 bp, synthetic construct
  misc_feature 1..42: note = synthetic
  source 1..42: mol_type = other DNA
gcgagatcaggcagctggttcgagaactggtacttcgatctc

SEQ ID NO: 88 - protein, 14 aa, synthetic construct
  REGION 1..14: note = synthetic
ARSGSWFENWYFDL

SEQ ID NO: 89 - DNA, 324 bp, synthetic construct
  misc_feature 1..324: note = synthetic
  source 1..324: mol_type = other DNA
gaaattgtgttgacgcagtctccaggcaccctgtctttgtctccaggggaaagagccaccctctcctgcagggccagtcagagtgttagcagcagctacttagcctggtaccagcagaaacctggccaggctcccaggctcctcatctatggtgcatccagcagggccactggcatcccagacaggttcagtggcagtgggtctgggacagacttcactctcaccatcagcagactggagcctgaagattttgcagtgtattactgtcagcagtatggtagctcaccttggacgttcggccaagggaccaaggtggaaatcaaa

SEQ ID NO: 90 - protein, 108 aa, synthetic construct
  REGION 1..108: note = synthetic
EIVLTQSPGTLSLSPGERATLSCRASQSVSSSYLAWYQQKPGQAPRLLIYGASSRATGIPDRFSGSGSGTDFTLTISRLEPEDFAVYYCQQYGSSPWTFGQGTKVEIK

SEQ ID NO: 91 - DNA, 21 bp, synthetic construct
  misc_feature 1..21: note = synthetic
  source 1..21: mol_type = other DNA
cagagtgttagcagcagctac

SEQ ID NO: 92 - protein, 7 aa, synthetic construct
  REGION 1..7: note = synthetic
QSVSSSY

SEQ ID NO: 93-94 - skipped (2 entries)

SEQ ID NO: 95 - DNA, 27 bp, synthetic construct
  misc_feature 1..27: note = synthetic
  source 1..27: mol_type = other DNA
cagcagtatggtagctcaccttggacg

SEQ ID NO: 96 - protein, 9 aa, synthetic construct
  REGION 1..9: note = synthetic
QQYGSSPWT

SEQ ID NO: 97 - DNA, 360 bp, synthetic construct
  misc_feature 1..360: note = synthetic
  source 1..360: mol_type = other DNA
caggtgcagctgcaggagtcgggcccaggactggtgaagccttcggagaccctgtccctcacctgcactgtctctggtggctccatcagtaattcctactggagctggatccggcagcccccagggaagggactggagtggattggatatgtctattcccgtgggaacaccaagtacaacccctccctcacgagtcgagtcaccatgtcatttgacacgtccaagaaccagttctccctgaaactgaggtctgtgaccgccgcagacacggccgtgtattactgtgcgagaagcagcagctggtacgaggactggtacttcgatctctggggccgtggcaccctggtcactgtctcctca

SEQ ID NO: 98 - protein, 120 aa, synthetic construct
  REGION 1..120: note = synthetic
QVQLQESGPGLVKPSETLSLTCTVSGGSISNSYWSWIRQPPGKGLEWIGYVYSRGNTKYNPSLTSRVTMSFDTSKNQFSLKLRSVTAADTAVYYCARSSSWYEDWYFDLWGRGTLVTVSS

SEQ ID NO: 99 - DNA, 24 bp, synthetic construct
  misc_feature 1..24: note = synthetic
  source 1..24: mol_type = other DNA
ggtggctccatcagtaattcctac

SEQ ID NO: 100 - protein, 8 aa, synthetic construct
  REGION 1..8: note = synthetic
GGSISNSY

SEQ ID NO: 101 - DNA, 21 bp, synthetic construct
  misc_feature 1..21: note = synthetic
  source 1..21: mol_type = other DNA
gtctattcccgtgggaacacc

SEQ ID NO: 102 - protein, 7 aa, synthetic construct
  REGION 1..7: note = synthetic
VYSRGNT

SEQ ID NO: 103 - DNA, 42 bp, synthetic construct
  misc_feature 1..42: note = synthetic
  source 1..42: mol_type = other DNA
gcgagaagcagcagctggtacgaggactggtacttcgatctc

SEQ ID NO: 104 - protein, 14 aa, synthetic construct
  REGION 1..14: note = synthetic
ARSSSWYEDWYFDL

SEQ ID NO: 105 - DNA, 354 bp, synthetic construct
  misc_feature 1..354: note = synthetic
  source 1..354: mol_type = other DNA
caggtgcagctacagcagtggggcgcagggctgtttaagccttcggagaccctgtccctcacctgcgatgtctatggtgggtccttcagaggttattattggagttggatccgccagcccccagggaaggggctggagtggattggggaaatcagttatagtggtttcaccaattacaacccgtccctcaagagtcgagtcatcatatcaatagatacgtccaagaaccagttctccctgaagatgagctctgtgaccgccgcggacacggctgtttattactgtgcgagagttacctatggttatgggacctttgattattggggccagggaaccctggtcaccgtctcctca

SEQ ID NO: 106 - protein, 118 aa, synthetic construct
  REGION 1..118: note = synthetic
QVQLQQWGAGLFKPSETLSLTCDVYGGSFRGYYWSWIRQPPGKGLEWIGEISYSGFTNYNPSLKSRVIISIDTSKNQFSLKMSSVTAADTAVYYCARVTYGYGTFDYWGQGTLVTVSS

SEQ ID NO: 107 - DNA, 24 bp, synthetic construct
  misc_feature 1..24: note = synthetic
  source 1..24: mol_type = other DNA
ggtgggtccttcagaggttattat

SEQ ID NO: 108 - protein, 8 aa, synthetic construct
  REGION 1..8: note = synthetic
GGSFRGYY

SEQ ID NO: 109 - DNA, 21 bp, synthetic construct
  misc_feature 1..21: note = synthetic
  source 1..21: mol_type = other DNA
atcagttatagtggtttcacc

SEQ ID NO: 110 - protein, 7 aa, synthetic construct
  REGION 1..7: note = synthetic
ISYSGFT

SEQ ID NO: 111 - DNA, 36 bp, synthetic construct
  misc_feature 1..36: note = synthetic
  source 1..36: mol_type = other DNA
gcgagagttacctatggttatgggacctttgattat

SEQ ID NO: 112 - protein, 12 aa, synthetic construct
  REGION 1..12: note = synthetic
ARVTYGYGTFDY

SEQ ID NO: 113 - protein, 1165 aa, Homo sapiens
  REGION 1..1165: note = hLEPR Accession No P48357
MICQKFCVVLLHWEFIYVITAFNLSYPITPWRFKLSCMPPNSTYDYFLLPAGLSKNTSNSNGHYETAVEPKFNSSGTHFSNLSKTTFHCCFRSEQDRNCSLCADNIEGKTFVSTVNSLVFQQIDANWNIQCWLKGDLKLFICYVESLFKNLFRNYNYKVHLLYVLPEVLEDSPLVPQKGSFQMVHCNCSVHECCECLVPVPTAKLNDTLLMCLKITSGGVIFQSPLMSVQPINMVKPDPPLGLHMEITDDGNLKISWSSPPLVPFPLQYQVKYSENSTTVIREADKIVSATSLLVDSILPGSSYEVQVRGKRLDGPGIWSDWSTPRVFTTQDVIYFPPKILTSVGSNVSFHCIYKKENKIVPSKEIVWWMNLAEKIPQSQYDVVSDHVSKVTFFNLNETKPRGKFTYDAVYCCNEHECHHRYAELYVIDVNINISCETDGYLTKMTCRWSTSTIQSLAESTLQLRYHRSSLYCSDIPSIHPISEPKDCYLQSDGFYECIFQPIFLLSGYTMWIRINHSLGSLDSPPTCVLPDSVVKPLPPSSVKAEITINIGLLKISWEKPVFPENNLQFQIRYGLSGKEVQWKMYEVYDAKSKSVSLPVPDLCAVYAVQVRCKRLDGLGYWSNWSNPAYTVVMDIKVPMRGPEFWRIINGDTMKKEKNVTLLWKPLMKNDSLCSVQRYVINHHTSCNGTWSEDVGNHTKFTFLWTEQAHTVTVLAINSIGASVANFNLTFSWPMSKVNIVQSLSAYPLNSSCVIVSWILSPSDYKLMYFIIEWKNLNEDGEIKWLRISSSVKKYYIHDHFIPIEKYQFSLYPIFMEGVGKPKIINSFTQDDIEKHQSDAGLYVIVPVIISSSILLLGTLLISHQRMKKLFWEDVPNPKNCSWAQGLNFQKPETFEHLFIKHTASVTCGPLLLEPETISEDISVDTSWKNKDEMMPTTVVSLLSTTDLEKGSVCISDQFNSVNFSEAEGTEVTYEDESQRQPFVKYATLISNSKPSETGEEQGLINSSVTKCFSSKNSPLKDSFSNSSWEIEAQAFFILSDQHPNIISPHLTFSEGLDELLKLEGNFPEENNDKKSIYYLGVTSIKKRESGVLLTDKSRVSCPFPAPCLFTDIRVLQDSCSHFVENNINLGTSSKKTFASYMPQFQTCSTQTHKIMENKMCDLTV

SEQ ID NO: 114 - protein, 846 aa, synthetic construct
  REGION 1..846: note = hLEPR.mmh aa 1-818: F22-D839 of P48357 aa 819-846: myc-myc-hexahistidine tag
FNLSYPITPWRFKLSCMPPNSTYDYFLLPAGLSKNTSNSNGHYETAVEPKFNSSGTHFSNLSKTTFHCCFRSEQDRNCSLCADNIEGKTFVSTVNSLVFQQIDANWNIQCWLKGDLKLFICYVESLFKNLFRNYNYKVHLLYVLPEVLEDSPLVPQKGSFQMVHCNCSVHECCECLVPVPTAKLNDTLLMCLKITSGGVIFQSPLMSVQPINMVKPDPPLGLHMEITDDGNLKISWSSPPLVPFPLQYQVKYSENSTTVIREADKIVSATSLLVDSILPGSSYEVQVRGKRLDGPGIWSDWSTPRVFTTQDVIYFPPKILTSVGSNVSFHCIYKKENKIVPSKEIVWWMNLAEKIPQSQYDVVSDHVSKVTFFNLNETKPRGKFTYDAVYCCNEHECHHRYAELYVIDVNINISCETDGYLTKMTCRWSTSTIQSLAESTLQLRYHRSSLYCSDIPSIHPISEPKDCYLQSDGFYECIFQPIFLLSGYTMWIRINHSLGSLDSPPTCVLPDSVVKPLPPSSVKAEITINIGLLKISWEKPVFPENNLQFQIRYGLSGKEVQWKMYEVYDAKSKSVSLPVPDLCAVYAVQVRCKRLDGLGYWSNWSNPAYTVVMDIKVPMRGPEFWRIINGDTMKKEKNVTLLWKPLMKNDSLCSVQRYVINHHTSCNGTWSEDVGNHTKFTFLWTEQAHTVTVLAINSIGASVANFNLTFSWPMSKVNIVQSLSAYPLNSSCVIVSWILSPSDYKLMYFIIEWKNLNEDGEIKWLRISSSVKKYYIHDHFIPIEKYQFSLYPIFMEGVGKPKIINSFTQDDIEKHQSDEQKLISEEDLGGEQKLISEEDLHHHHHH

SEQ ID NO: 115 - protein, 1051 aa, synthetic construct
  REGION 1..1051: note = hLEPR.mFc aa 1-818: F22-D839 of P48357 aa 819-1051: mouse IgG2a (E98-K330 of P01863)
FNLSYPITPWRFKLSCMPPNSTYDYFLLPAGLSKNTSNSNGHYETAVEPKFNSSGTHFSNLSKTTFHCCFRSEQDRNCSLCADNIEGKTFVSTVNSLVFQQIDANWNIQCWLKGDLKLFICYVESLFKNLFRNYNYKVHLLYVLPEVLEDSPLVPQKGSFQMVHCNCSVHECCECLVPVPTAKLNDTLLMCLKITSGGVIFQSPLMSVQPINMVKPDPPLGLHMEITDDGNLKISWSSPPLVPFPLQYQVKYSENSTTVIREADKIVSATSLLVDSILPGSSYEVQVRGKRLDGPGIWSDWSTPRVFTTQDVIYFPPKILTSVGSNVSFHCIYKKENKIVPSKEIVWWMNLAEKIPQSQYDVVSDHVSKVTFFNLNETKPRGKFTYDAVYCCNEHECHHRYAELYVIDVNINISCETDGYLTKMTCRWSTSTIQSLAESTLQLRYHRSSLYCSDIPSIHPISEPKDCYLQSDGFYECIFQPIFLLSGYTMWIRINHSLGSLDSPPTCVLPDSVVKPLPPSSVKAEITINIGLLKISWEKPVFPENNLQFQIRYGLSGKEVQWKMYEVYDAKSKSVSLPVPDLCAVYAVQVRCKRLDGLGYWSNWSNPAYTVVMDIKVPMRGPEFWRIINGDTMKKEKNVTLLWKPLMKNDSLCSVQRYVINHHTSCNGTWSEDVGNHTKFTFLWTEQAHTVTVLAINSIGASVANFNLTFSWPMSKVNIVQSLSAYPLNSSCVIVSWILSPSDYKLMYFIIEWKNLNEDGEIKWLRISSSVKKYYIHDHFIPIEKYQFSLYPIFMEGVGKPKIINSFTQDDIEKHQSDEPRGPTIKPCPPCKCPAPNLLGGPSVFIFPPKIKDVLMISLSPIVTCVVVDVSEDDPDVQISWFVNNVEVHTAQTQTHREDYNSTLRVVSALPIQHQDWMSGKEFKCKVNNKDLPAPIERTISKPKGSVRAPQVYVLPPPEEEMTKKQVTLTCMVTDFMPEDIYVEWTNNGKTELNYKNTEPVLDSDGSYFMYSKLRVEKKNWVERNSYSCSVVHEGLHNHHTTKSFSRTPGK

SEQ ID NO: 116 - protein, 1045 aa, synthetic construct
  REGION 1..1045: note = hLEPR.hFc aa 1-818: F22-D839 of P48357 aa 819-1045: human IgG1 tag (D104-K330 of P01857)
FNLSYPITPWRFKLSCMPPNSTYDYFLLPAGLSKNTSNSNGHYETAVEPKFNSSGTHFSNLSKTTFHCCFRSEQDRNCSLCADNIEGKTFVSTVNSLVFQQIDANWNIQCWLKGDLKLFICYVESLFKNLFRNYNYKVHLLYVLPEVLEDSPLVPQKGSFQMVHCNCSVHECCECLVPVPTAKLNDTLLMCLKITSGGVIFQSPLMSVQPINMVKPDPPLGLHMEITDDGNLKISWSSPPLVPFPLQYQVKYSENSTTVIREADKIVSATSLLVDSILPGSSYEVQVRGKRLDGPGIWSDWSTPRVFTTQDVIYFPPKILTSVGSNVSFHCIYKKENKIVPSKEIVWWMNLAEKIPQSQYDVVSDHVSKVTFFNLNETKPRGKFTYDAVYCCNEHECHHRYAELYVIDVNINISCETDGYLTKMTCRWSTSTIQSLAESTLQLRYHRSSLYCSDIPSIHPISEPKDCYLQSDGFYECIFQPIFLLSGYTMWIRINHSLGSLDSPPTCVLPDSVVKPLPPSSVKAEITINIGLLKISWEKPVFPENNLQFQIRYGLSGKEVQWKMYEVYDAKSKSVSLPVPDLCAVYAVQVRCKRLDGLGYWSNWSNPAYTVVMDIKVPMRGPEFWRIINGDTMKKEKNVTLLWKPLMKNDSLCSVQRYVINHHTSCNGTWSEDVGNHTKFTFLWTEQAHTVTVLAINSIGASVANFNLTFSWPMSKVNIVQSLSAYPLNSSCVIVSWILSPSDYKLMYFIIEWKNLNEDGEIKWLRISSSVKKYYIHDHFIPIEKYQFSLYPIFMEGVGKPKIINSFTQDDIEKHQSDDKTHTCPPCPAPELLGGPSVFLFPPKPKDTLMISRTPEVTCVVVDVSHEDPEVKFNWYVDGVEVHNAKTKPREEQYNSTYRVVSVLTVLHQDWLNGKEYKCKVSNKALPAPIEKTISKAKGQPREPQVYTLPPSRDELTKNQVSLTCLVKGFYPSDIAVEWESNGQPENNYKTTPPVLDSDGSFFLYSKLTVDKSRWQQGNVFSCSVMHEALHNHYTQKSLSLSPGK

SEQ ID NO: 117 - protein, 844 aa, synthetic construct
  REGION 1..844: note = MfLEPR.mmh aa 1-816: Macaca fascicularis F22-D837 with a T827A substitution from XP_005543194.1 aa 817-844: myc-myc-hexahistidine tag
FNLSYPITPWRFKLSCMPPNSTYDYFLLPAGLSKNTSNLNGHYETAVEFNSSDTHFSNLSKTTFHCCFRSEQDRNCSLCADNIEGKTFVSTVNSSVFQQMGANWNIQCWLKGDLKLFICYVESLFKNPFKNYKHKVHLLYVLPEVLEDSPLVPQKGSFQMVHCNCSVHERCECLVPVPTAKLNDTLLMCLKITSGGVIFQSPLMSVQPINMVKPDPPLGLRMEITDDGNLKISWSSPPLVPFPLQYEVKYSENSTTVIREADKIVSATSLLVDGILPGSSYEVQVRGKRLDGPGIWSDWSTPHVFTTQDVIYFPPKILTSVGSNVSFHCIYKNENKIVSSKKIVWWMNLAEKIPQSQYDVVSDHVSKVTFFNLNETKPRGKFTYDAVYCCNEHECHHRYAELYVIDVNINISCETDGHLTKMTCRWSTNTIQSLAGSTLQLRYRRSSLYCFDIPSIHPISKPKDCYLQSDGFYECVFQPIFLLSGYTMWIRINHPLGSLDSPPTCVLPDSVVKPLPPSSVKAEIIKNIGLLKISWEKPVFPENNLQFQIRYGLSGKEIQWKMYDVYDAKSKSVSLPVPDFCAVYAVQVRCKRSDGLGLWSNWSNPAYTVVMDIKVPMRGPEFWRIINGDTMKKEKNVTLLWKPLMKNDSLCSVQRYVINHHTSCNGTWSEDVGNHTKFTFLWTEQAHTVTVLAINSIGASVANFNLTFSWPMSKVNIVQSLSAYPLNSSCVILSWILSPSDYKLMYFIIEWKNLNEDGEIKWLRISSSVKKYYIHDHFIPIEKYQFSLYPIFMEGVGKPKIINSFAQDNTEKHQNDEQKLISEEDLGGEQKLISEEDLHHHHHH

SEQ ID NO: 118 - protein, 846 aa, synthetic construct
  REGION 1..846: note = mLEPR.mmh aa 1-818: Mouse LEPR (L22-G839 of NP_666258.2) aa 817-846: myc-myc-hexahistidine tag
LNLAYPISPWKFKLFCGPPNTTDDSFLSPAGAPNNASALKGASEAIVEAKFNSSGIYVPELSKTVFHCCFGNEQGQNCSALTDNTEGKTLASVVKASVFRQLGVNWDIECWMKGDLTLFICHMEPLPKNPFKNYDSKVHLLYDLPEVIDDSPLPPLKDSFQTVQCNCSLRGCECHVPVPRAKLNYALLMYLEITSAGVSFQSPLMSLQPMLVVKPDPPLGLHMEVTDDGNLKISWDSQTMAPFPLQYQVKYLENSTIVREAAEIVSATSLLVDSVLPGSSYEVQVRSKRLDGSGVWSDWSSPQVFTTQDVVYFPPKILTSVGSNASFHCIYKNENQIISSKQIVWWRNLAEKIPEIQYSIVSDRVSKVTFSNLKATRPRGKFTYDAVYCCNEQACHHRYAELYVIDVNINISCETDGYLTKMTCRWSPSTIQSLVGSTVQLRYHRRSLYCPDSPSIHPTSEPKNCVLQRDGFYECVFQPIFLLSGYTMWIRINHSLGSLDSPPTCVLPDSVVKPLPPSNVKAEITVNTGLLKVSWEKPVFPENNLQFQIRYGLSGKEIQWKTHEVFDAKSKSASLLVSDLCAVYVVQVRCRRLDGLGYWSNWSSPAYTLVMDVKVPMRGPEFWRKMDGDVTKKERNVTLLWKPLTKNDSLCSVRRYVVKHRTAHNGTWSEDVGNRTNLTFLWTEPAHTVTVLAVNSLGASLVNFNLTFSWPMSKVSAVESLSAYPLSSSCVILSWTLSPDDYSLLYLVIEWKILNEDDGMKWLRIPSNVKKFYIHDNFIPIEKYQFSLYPVFMEGVGKPKIINGFTKDAIDKQQNDAGEQKLISEEDLGGEQKLISEEDLHHHHHH

SEQ ID NO: 119 - protein, 846 aa, synthetic construct
  REGION 1..846: note = rLEPR.mmh aa 1-818: Rat LEPR (L22-G839 of NP_036728.1) aa 819-846: myc-myc-hexahistidine tag
LNLAYPTSPWRFKLFCAPPSTTDDSFLSPAGVPNNTSSLKGASEALVEAKFNSTGIYVSELSKTIFHCCFGNEQGQNCSALTGNTEGKTLASVVKPLVFRQLGVNWDIECWMKGDLTLFICHMEPLLKNPFKNYDSKVHLLYDLPEVIDDLPLPPLKDSFQTVQCNCSVRECECHVPVPRAKVNYALLMYLEITSAGVSFQSPLMSLQPMLVVKPDPPLGLRMEVTDDGNLKISWDSQTKAPFPLQYQVKYLENSTIVREAAEIVSDTSLLVDSVLPGSSYEVQVRSKRLDGSGVWSDWSLPQLFTTQDVMYFPPKILTSVGSNASFCCIYKNENQTISSKQIVWWMNLAEKIPETQYNTVSDHISKVTFSNLKATRPRGKFTYDAVYCCNEQACHHRYAELYVIDVNINISCETDGYLTKMTCRWSPSTIQSLVGSTVQLRYHRRSLYCPDNPSIRPTSELKNCVLQTDGFYECVFQPIFLLSGYTMWIRINHSLGSLDSPPTCVLPDSVVKPLPPSNVKAEITINTGLLKVSWEKPVFPENNLQFQIRYGLNGKEIQWKTHEVFDAKSKSASLPVSDLCAVYVVQVRCRRLDGLGYWSNWSSPAYTLVMDVKVPMRGPEFWRIMDGDITKKERNVTLLWKPLMKNDSLCSVRRYVVKHRTAHNGTWSQDVGNQTNLTFLWAESAHTVTVLAINSIGASLVNFNLTFSWPMSKVNAVQSLSAYPLSSSCVILSWTLSPNDYSLLYLVIEWKNLNDDDGMKWLRIPSNVNKYYIHDNFIPIEKYQFSLYPVFMEGVGKPKIINGFTKDDIAKQQNDAGEQKLISEEDLGGEQKLISEEDLHHHHHH

SEQ ID NO: 120 - protein, 1045 aa, synthetic construct
  REGION 1..1045: note = mLEPR.hFc aa 1-818: Mouse LEPR (L22-G839 of NP_666258.2) aa 819-1045: human IgG1 tag (D104-K330 of P01857)
LNLAYPISPWKFKLFCGPPNTTDDSFLSPAGAPNNASALKGASEAIVEAKFNSSGIYVPELSKTVFHCCFGNEQGQNCSALTDNTEGKTLASVVKASVFRQLGVNWDIECWMKGDLTLFICHMEPLPKNPFKNYDSKVHLLYDLPEVIDDSPLPPLKDSFQTVQCNCSLRGCECHVPVPRAKLNYALLMYLEITSAGVSFQSPLMSLQPMLVVKPDPPLGLHMEVTDDGNLKISWDSQTMAPFPLQYQVKYLENSTIVREAAEIVSATSLLVDSVLPGSSYEVQVRSKRLDGSGVWSDWSSPQVFTTQDVVYFPPKILTSVGSNASFHCIYKNENQIISSKQIVWWRNLAEKIPEIQYSIVSDRVSKVTFSNLKATRPRGKFTYDAVYCCNEQACHHRYAELYVIDVNINISCETDGYLTKMTCRWSPSTIQSLVGSTVQLRYHRRSLYCPDSPSIHPTSEPKNCVLQRDGFYECVFQPIFLLSGYTMWIRINHSLGSLDSPPTCVLPDSVVKPLPPSNVKAEITVNTGLLKVSWEKPVFPENNLQFQIRYGLSGKEIQWKTHEVFDAKSKSASLLVSDLCAVYVVQVRCRRLDGLGYWSNWSSPAYTLVMDVKVPMRGPEFWRKMDGDVTKKERNVTLLWKPLTKNDSLCSVRRYVVKHRTAHNGTWSEDVGNRTNLTFLWTEPAHTVTVLAVNSLGASLVNFNLTFSWPMSKVSAVESLSAYPLSSSCVILSWTLSPDDYSLLYLVIEWKILNEDDGMKWLRIPSNVKKFYIHDNFIPIEKYQFSLYPVFMEGVGKPKIINGFTKDAIDKQQNDAGDKTHTCPPCPAPELLGGPSVFLFPPKPKDTLMISRTPEVTCVVVDVSHEDPEVKFNWYVDGVEVHNAKTKPREEQYNSTYRVVSVLTVLHQDWLNGKEYKCKVSNKALPAPIEKTISKAKGQPREPQVYTLPPSRDELTKNQVSLTCLVKGFYPSDIAVEWESNGQPENNYKTTPPVLDSDGSFFLYSKLTVDKSRWQQGNVFSCSVMHEALHNHYTQKSLSLSPGK